European Patent Specification EP 3 677 592 B1, published July 17, 2024. Title: MODIFIED HSV GD PROTEIN AND VACCINE CONTAINING SAME. Applicant: KM Biologics Co., Ltd. The sequence listing filed with the application follows.

SEQUENCE LISTING (34 sequences)

SEQ ID NO: 1 - protein, 315 aa, Herpes simplex virus
  HSV gD1-315
KYALADPSLKMADPNRFRGKNLPVLDQLTDPPGVKRVYHIQPSLEDPFQPPSIPITVYYAVLERACRSVLLHAPSEAPQIVRGASDEARKHTYNLTIAWYRMGDNCAIPITVMEYTECPYNKSLGVCPIRTQPRWSYYDSFSAVSEDNLGFLMHAPAFETAGTYLRLVKINDWTEITQFILEHRARASCKYALPLRIPPAACLTSKAYQQGVTVDSIGMLPRFIPENQRTVALYSLKIAGWHGPKPPYTSTLLPPELSDTTNATQPELVPEDPEDSALLEDPAGTVSSQIPPNWHIPSIQDVAPHHAPAAPSNPG

SEQ ID NO: 2 - protein, 394 aa, Herpes simplex virus-1
MGGAAARLGAVILFVVIVGLHGVRGKYALADASLKMADPNRFRGKDLPVLDQLTDPPGVRRVYHIQAGLPDPFQPPSLPITVYYAVLERACRSVLLNAPSEAPQIVRGASEDVRKQPYNLTIAWFRMGGNCAIPITVMEYTECSYNKSLGACPIRTQPRWNYYDSFSAVSEDNLGFLMHAPAFETAGTYLRLVKINDWTEITQFILEHRAKGSCKYALPLRIPPSACLSPQAYQQGVTVDSIGMLPRFIPENQRTVAVYSLKIAGWHGPKAPYTSTLLPPELSETPNATQPELAPEDPEDSALLEDPVGTVAPQIPPNWHIPSIQDAATPYHPPATPNNMGLIAGAVGGSLLAALVICGIVYWMHRRTRKAPKRIRLPHIREDDQPSSHQPLFY

SEQ ID NO: 3 - protein, 393 aa, Herpes simplex virus-2
MGRLTSGVGTAALLVVAVGLRVVCAKYALADPSLKMADPNRFRGKNLPVLDQLTDPPGVKRVYHIQPSLEDPFQPPSIPITVYYAVLERACRSVLLHAPSEAPQIVRGASDEARKHTYNLTIAWYRMGDNCAIPITVMEYTECPYNKSLGVCPIRTQPRWSYYDSFSAVSEDNLGFLMHAPAFETAGTYLRLVKINDWTEITQFILEHRARASCKYALPLRIPPAACLTSKAYQQGVTVDSIGMLPRFIPENQRTVALYSLKIAGWHGPKPPYTSTLLPPELSDTTNATQPELVPEDPEDSALLEDPAGTVSSQIPPNWHIPSIQDVAPHHAPAAPSNPGLIIGALAGSTLAVLVIGGIAFWVRRRAQMAPKRLRLPHIRDDDAPPSHQPLFY

SEQ ID NO: 4 - protein, 15 aa, Herpes simplex virus-2
KRVYHIQPSLEDPFQ

SEQ ID NO: 5 - protein, 17 aa, Herpes simplex virus-2
ITVYYAVLERACRSVLL

SEQ ID NO: 6 - protein, 22 aa, Herpes simplex virus-2
INDWTEITQFILEHRARASCKY

SEQ ID NO: 7 - protein, 16 aa, Herpes simplex virus-2
PGLIIGALAGSTLAVL

SEQ ID NO: 8 - protein, 17 aa, Herpes simplex virus-2
IAFWVRRRAQMAPKPLR

SEQ ID NO: 9 - protein, 5 aa, Artificial Sequence
  No.82 H-CDR1
GYAIN

SEQ ID NO: 10 - protein, 16 aa, Artificial Sequence
  No.82 H-CDR2
GIMPIFGTSNYAQKFQ

SEQ ID NO: 11 - protein, 16 aa, Artificial Sequence
  No.82 H-CDR3
DWGAPLEKGAGSPFDV

SEQ ID NO: 12 - protein, 12 aa, Artificial Sequence
  No.82 L-CDR1
RASQSVSSSYLA

SEQ ID NO: 13 - protein, 7 aa, Artificial Sequence
  No.82 L-CDR2
GASSRAT

SEQ ID NO: 14 - protein, 9 aa, Artificial Sequence
  No.82 L-CDR3
QQYGSSPRS

SEQ ID NO: 15 - DNA, 27 bp, Artificial Sequence
  SC-A-Fw
cgggccaatgcctcctgcaagtacgct

SEQ ID NO: 16 - DNA, 27 bp, Artificial Sequence
  SC-A-Re
ggaggcattggcccggtgctccaggat

SEQ ID NO: 17 - DNA, 33 bp, Artificial Sequence
  SC-B-Fw
gggtggaatggcaccaagcccccgtacaccagc

SEQ ID NO: 18 - DNA, 33 bp, Artificial Sequence
  SC-B-Re
gggcttggtgccattccacccggcgatttttaa

SEQ ID NO: 19 - DNA, 33 bp, Artificial Sequence
  SC-D-Fw
catgccaattcgaccgccccccagatcgtgcgc

SEQ ID NO: 20 - DNA, 33 bp, Artificial Sequence
  SC-D-Re
gggggcggtcgaattggcatgtaggagcacgct

SEQ ID NO: 21 - DNA, 33 bp, Artificial Sequence
  SC-E-Fw
cgcatgaatgacacctgcgctatccccatcacg

SEQ ID NO: 22 - DNA, 33 bp, Artificial Sequence
  SC-E-Re
agcgcaggtgtcattcatgcgataccaggcgat

SEQ ID NO: 23 - DNA, 33 bp, Artificial Sequence
  SC-F-Fw
ttccagaatgcaagcatcccgatcactgtgtac

SEQ ID NO: 24 - DNA, 33 bp, Artificial Sequence
  SC-F-Re
cgggatgcttgcattctggaacgggtcctccag

SEQ ID NO: 25 - DNA, 33 bp, Artificial Sequence
  SC-H-Fw
ctccccaatcgcacgcccccggcagcgtgcctc

SEQ ID NO: 26 - DNA, 33 bp, Artificial Sequence
  SC-H-Re
cgggggcgtgcgattggggagagcgtacttgca

SEQ ID NO: 27 - DNA, 27 bp, Artificial Sequence
  SC-K-Fw
agcatcaatatcactgtgtactacgca

SEQ ID NO: 28 - DNA, 27 bp, Artificial Sequence
  SC-K-Re
agtgatattgatgctggggggctggaa

SEQ ID NO: 29 - DNA, 33 bp, Artificial Sequence
  SC-L-Fw
ggggctaatgacaccgcccgaaagcacacgtac

SEQ ID NO: 30 - DNA, 33 bp, Artificial Sequence
  SC-L-Re
tcgggcggtgtcattagccccgcgcacgatctg

SEQ ID NO: 31 - DNA, 27 bp, Artificial Sequence
  SC-M-Fw
ataaacaattggacggagatcacacaa

SEQ ID NO: 32 - DNA, 27 bp, Artificial Sequence
  SC-M-Re
cgtccaattgtttatcttcactagccg

SEQ ID NO: 33 - DNA, 1180 bp, Herpes simplex virus-2
atggggcgtttgacctccggcgtcgggacggcggccctgctagttgtcgcggtgggactccgcgtcgtctgcgccaaatacgccttagcagacccctcgcttaagatggccgatcccaatcgatttcgcgggaagaaccttccggttttggaccagctgaccgacccccccggggtgaagcgtgtttaccacattcagccgagcctggaggacccgttccagccccccagcatcccgatcactgtgtactacgcagtgctggaacgtgcctgccgcagcgtgctcctacatgccccatcggaggccccccagatcgtgcgcggggcttcggacgaggcccgaaagcacacgtacaacctgaccatcgcctggtatcgcatgggagacaattgcgctatccccatcacggttatggaatacaccgagtgcccctacaacaagtcgttgggggtctgccccatccgaacgcagccccgctggagctactatgacagctttagcgccgtcagcgaggataacctgggattcctgatgcacgcccccgccttcgagaccgcgggtacgtacctgcggctagtgaagataaacgactggacggagatcacacaatttatcctggagcaccgggcccgcgcctcctgcaagtacgctctccccctgcgcatccccccggcagcgtgcctcacctcgaaggcctaccaacagggcgtgacggtcgacagcatcgggatgctcccccgctttatccccgaaaaccagcgcaccgtcgccctatacagcttaaaaatcgccgggtggcacggccccaagcccccgtacaccagcaccctgctgccgccggagctgtccgacaccaccaacgccacgcaacccgaactcgttccggaagaccccgaggactcggccctcttagaggatcccgccgggacggtgtcttcgcagatccccccaaactggcacatcccgtcgatccaggacgtcgcgccgcaccacgcccccgccgcccccagcaacccgggcctgatcatcggcgcgctggccggcagtaccctggcggtgctggtcatcggcggtattgcgttttgggtacgccgccgcgctcagatggcccccaagcgcctacgtctcccccacatccgggatgacgacgcgcccccctcgcaccagccattgttttact

SEQ ID NO: 34 - protein, 5 aa, Artificial Sequence
  Linker
GPGPG